European Patent Application EP 4 169 526 A1, published April 26, 2023. Title: Arginase and Argininosuccinate Synthase for cancer therapy. Applicant: Kyon Biotech AG. The sequence listing filed with the application follows.

SEQUENCE LISTING (2 sequences)

SEQ ID NO: 1 - protein, 331 aa, Artificial Sequence
  modified ARG1
MGHHHHHHGSSAKSRTIGIIGAPFSKGQPRGGVEEGPTVLRKAGLLEKLKEQECDVKDYGDLPFADIPNDSPFQIVKNPRSVGKASEQLAGKVAEVKKNGRISLVLGGDHSLAIGSISGHARVHPDLGVIWVDAHTDINTPLTTTSGNLHGQPVSFLLKELKGKIPDVPGFSWVTPCISAKDIVYIGLRDVDPGEHYILKTLGIKYFSMTEVDRLGIGKVMEETLSYLLGRKKRPIHLSFDVDGLDPSFTPATGTPVVGGLTYREGLYITEEIYKTGLLSGLDIMEVNPSLGKTPEEVTRTVNTAVAITLACFGLAREGNHKPIDYLNPPK

SEQ ID NO: 2 - protein, 424 aa, Artificial Sequence
  modified ASS1
MGHHHHHHHHGSGSSKGSVVLAYSGGLDTSCILVWLKEQGYDVIAYLANIGQKEDFEEARKKALKLGAKKVFIEDVSREFVEEFIWPAIQSSALYEDRYLLGTSLARPCIARKQVEIAQREGAKYVSHGATGKGNDQVRFELSCYSLAPQIKVIAPWRMPEFYNRFKGRNDLMEYAKQHGIPIPVTPKNPWSMDENLMHISYEAGILENPKNQAPPGLYTKTQDPAKAPNTPDILEIEFKKGVPVKVTNVKDGTTHQTSLELFMYLNEVAGKHGVGRIDIVENRFIGMKSRGIYETPAGTILYHAHLDIEAFTMDREVRKIKQGLGLKFAELVYTGFWHSPECEFVRHCIAKSQERVEGKVQVSVLKGQVYILGRESPLSLYNEELVSMNVQGDYEPTDATGFININSLRLKEYHRLQSKVTAK